European Patent Application EP 4 534 670 A1, published April 9, 2025. Title: Composition for regulating splicing of polybromo 1 mRNA comprising splicing-switch oligonucleotide as effective component. Applicant: The Industry & Academic Cooperation in Chungnam National University (IAC). Application KR. The sequence listing filed with the application follows.

SEQUENCE LISTING (5 sequences)

SEQ ID NO: 1 - RNA, 21 nt, synthetic construct
  source 1..21: mol_type = other RNA
gccttgaaggacacaaatttc

SEQ ID NO: 2 - RNA, 24 nt, synthetic construct
  source 1..24: mol_type = other RNA
cacccatcatgccttgaaggacac

SEQ ID NO: 3 - RNA, 23 nt, synthetic construct
  source 1..23: mol_type = other RNA
tgcattcgccctcttaatgggga

SEQ ID NO: 4 - DNA, 15 bp, synthetic construct
  source 1..15: mol_type = other DNA
gtagcccaccaagac

SEQ ID NO: 5 - DNA, 17 bp, synthetic construct
  source 1..17: mol_type = other DNA
gctggagtcaccatagg